European Patent Application EP 4 335 868 A1, published March 13, 2024. Title: FC MUTANT WITH ALTERED BINDING TO FC RECEPTOR. Applicant: Innovent Biologics (Suzhou) Co., Ltd. The sequence listing filed with the application follows.

SEQUENCE LISTING (34 sequences)

SEQ ID NO: 1 - protein, 448 aa, Artificial sequence
  Synthesized
QVQLVQSGAEVKKPGSSVKVSCKASGYSFSSYNIHWVRQAPGQGLEWMGYIAPFQGDSRYNQKFKGRVTITADKSTSTAYMELSSLRSEDTAVYYCARLNRGNSLDYWGQGTLVTVSSASTKGPSVFPLAPSSKSTSGGTAALGCLVKDYFPEPVTVSWNSGALTSGVHTFPAVLQSSGLYSLSSVVTVPSSSLGTQTYICNVNHKPSNTKVDKKVEPKSCDKTHTCPPCPAPELLGGPSVFLFPPKPKDTLMISRTPEVTCVVVDVSHEDPEVKFNWYVDGVEVHNAKTKPREEQYNSTYRVVSVLTVLHQDWLNGKEYKCKVSNKALPAPIEKTISKAKGQPREPQVYTLPPSREEMTKNQVSLTCLVKGFYPSDIAVEWESNGQPENNYKTTPPVLDSDGSFFLYSKLTVDKSRWQQGNVFSCSVMHEALHNHYTQKSLSLSPGK

SEQ ID NO: 2 - protein, 447 aa, Artificial sequence
  Synthesized
QVQLVQSGAEVKKPGSSVKVSCKASGYSFSSYNIHWVRQAPGQGLEWMGYIAPFQGDSRYNQKFKGRVTITADKSTSTAYMELSSLRSEDTAVYYCARLNRGNSLDYWGQGTLVTVSSASTKGPSVFPLAPSSKSTSGGTAALGCLVKDYFPEPVTVSWNSGALTSGVHTFPAVLQSSGLYSLSSVVTVPSSSLGTQTYICNVNHKPSNTKVDKKVEPKSCDKTHTCPPCPAPELLGGPSVFLFPPKPKDTLMISRTPEVTCVVVDVSHEDPEVKFNWYVDGVEVHNAKTKPREEQYNSTYRVVSVLTVLHQDWLNGKEYKCKVSNKALAPIEKTISKAKGQPREPQVYTLPPSREEMTKNQVSLTCLVKGFYPSDIAVEWESNGQPENNYKTTPPVLDSDGSFFLYSKLTVDKSRWQQGNVFSCSVMHEALHNHYTQKSLSLSPGK

SEQ ID NO: 3 - protein, 447 aa, Artificial sequence
  Synthesized
QVQLVQSGAEVKKPGSSVKVSCKASGYSFSSYNIHWVRQAPGQGLEWMGYIAPFQGDSRYNQKFKGRVTITADKSTSTAYMELSSLRSEDTAVYYCARLNRGNSLDYWGQGTLVTVSSASTKGPSVFPLAPSSKSTSGGTAALGCLVKDYFPEPVTVSWNSGALTSGVHTFPAVLQSSGLYSLSSVVTVPSSSLGTQTYICNVNHKPSNTKVDKKVEPKSCDKTHTCPPCPAPELLGGPSVFLFPPKPKDTLMISRTPEVTCVVVDVSHEDPEVKFNWYVDGVEVHNAKTKPREEQYNSTYRVVSVLTVLHQDWLNGKEYKCKVSNKALGPIEKTISKAKGQPREPQVYTLPPSREEMTKNQVSLTCLVKGFYPSDIAVEWESNGQPENNYKTTPPVLDSDGSFFLYSKLTVDKSRWQQGNVFSCSVMHEALHNHYTQKSLSLSPGK

SEQ ID NO: 4 - protein, 446 aa, Artificial sequence
  Synthesized
QVQLVQSGAEVKKPGSSVKVSCKASGYSFSSYNIHWVRQAPGQGLEWMGYIAPFQGDSRYNQKFKGRVTITADKSTSTAYMELSSLRSEDTAVYYCARLNRGNSLDYWGQGTLVTVSSASTKGPSVFPLAPSSKSTSGGTAALGCLVKDYFPEPVTVSWNSGALTSGVHTFPAVLQSSGLYSLSSVVTVPSSSLGTQTYICNVNHKPSNTKVDKKVEPKSCDKTHTCPPCPAPELLGGPSVFLFPPKPKDTLMISRTPEVTCVVVDVSHEDPEVKFNWYVDGVEVHNAKTKPREEQYNSTYRVVSVLTVLHQDWLNGKEYKCKVSNKALPIEKTISKAKGQPREPQVYTLPPSREEMTKNQVSLTCLVKGFYPSDIAVEWESNGQPENNYKTTPPVLDSDGSFFLYSKLTVDKSRWQQGNVFSCSVMHEALHNHYTQKSLSLSPGK

SEQ ID NO: 5 - protein, 448 aa, Artificial sequence
  Synthesized
QVQLVQSGAEVKKPGSSVKVSCKASGYSFSSYNIHWVRQAPGQGLEWMGYIAPFQGDSRYNQKFKGRVTITADKSTSTAYMELSSLRSEDTAVYYCARLNRGNSLDYWGQGTLVTVSSASTKGPSVFPLAPSSKSTSGGTAALGCLVKDYFPEPVTVSWNSGALTSGVHTFPAVLQSSGLYSLSSVVTVPSSSLGTQTYICNVNHKPSNTKVDKKVEPKSCDKTHTCPPCPAPEAAGGPSVFLFPPKPKDTLMISRTPEVTCVVVDVSHEDPEVKFNWYVDGVEVHNAKTKPREEQYNSTYRVVSVLTVLHQDWLNGKEYKCKVSNKALPAPIEKTISKAKGQPREPQVYTLPPSREEMTKNQVSLTCLVKGFYPSDIAVEWESNGQPENNYKTTPPVLDSDGSFFLYSKLTVDKSRWQQGNVFSCSVMHEALHNHYTQKSLSLSPGK

SEQ ID NO: 6 - protein, 447 aa, Artificial sequence
  Synthesized
QVQLVQSGAEVKKPGSSVKVSCKASGYSFSSYNIHWVRQAPGQGLEWMGYIAPFQGDSRYNQKFKGRVTITADKSTSTAYMELSSLRSEDTAVYYCARLNRGNSLDYWGQGTLVTVSSASTKGPSVFPLAPSSKSTSGGTAALGCLVKDYFPEPVTVSWNSGALTSGVHTFPAVLQSSGLYSLSSVVTVPSSSLGTQTYICNVNHKPSNTKVDKKVEPKSCDKTHTCPPCPAPEAAGGPSVFLFPPKPKDTLMISRTPEVTCVVVDVSHEDPEVKFNWYVDGVEVHNAKTKPREEQYNSTYRVVSVLTVLHQDWLNGKEYKCKVSNKALAPIEKTISKAKGQPREPQVYTLPPSREEMTKNQVSLTCLVKGFYPSDIAVEWESNGQPENNYKTTPPVLDSDGSFFLYSKLTVDKSRWQQGNVFSCSVMHEALHNHYTQKSLSLSPGK

SEQ ID NO: 7 - protein, 447 aa, Artificial sequence
  Synthesized
QVQLVQSGAEVKKPGSSVKVSCKASGYSFSSYNIHWVRQAPGQGLEWMGYIAPFQGDSRYNQKFKGRVTITADKSTSTAYMELSSLRSEDTAVYYCARLNRGNSLDYWGQGTLVTVSSASTKGPSVFPLAPSSKSTSGGTAALGCLVKDYFPEPVTVSWNSGALTSGVHTFPAVLQSSGLYSLSSVVTVPSSSLGTQTYICNVNHKPSNTKVDKKVEPKSCDKTHTCPPCPAPEAAGGPSVFLFPPKPKDTLMISRTPEVTCVVVDVSHEDPEVKFNWYVDGVEVHNAKTKPREEQYNSTYRVVSVLTVLHQDWLNGKEYKCKVSNKALGPIEKTISKAKGQPREPQVYTLPPSREEMTKNQVSLTCLVKGFYPSDIAVEWESNGQPENNYKTTPPVLDSDGSFFLYSKLTVDKSRWQQGNVFSCSVMHEALHNHYTQKSLSLSPGK

SEQ ID NO: 8 - protein, 446 aa, Artificial sequence
  Synthesized
QVQLVQSGAEVKKPGSSVKVSCKASGYSFSSYNIHWVRQAPGQGLEWMGYIAPFQGDSRYNQKFKGRVTITADKSTSTAYMELSSLRSEDTAVYYCARLNRGNSLDYWGQGTLVTVSSASTKGPSVFPLAPSSKSTSGGTAALGCLVKDYFPEPVTVSWNSGALTSGVHTFPAVLQSSGLYSLSSVVTVPSSSLGTQTYICNVNHKPSNTKVDKKVEPKSCDKTHTCPPCPAPEAAGGPSVFLFPPKPKDTLMISRTPEVTCVVVDVSHEDPEVKFNWYVDGVEVHNAKTKPREEQYNSTYRVVSVLTVLHQDWLNGKEYKCKVSNKALPIEKTISKAKGQPREPQVYTLPPSREEMTKNQVSLTCLVKGFYPSDIAVEWESNGQPENNYKTTPPVLDSDGSFFLYSKLTVDKSRWQQGNVFSCSVMHEALHNHYTQKSLSLSPGK

SEQ ID NO: 9 - protein, 220 aa, Artificial sequence
  Synthesized
DIVMTQSPDSLAVSLGERATINCKSSQSLFNSGNQRNYLTWYQQKPGQPPKLLIYWASTRESGVPDRFSGSGSGTDFTLTISSLQAEDVAVYYCQNNYIYPLTFGGGTKVEIKRTVAAPSVFIFPPSDEQLKSGTASVVCLLNNFYPREAKVQWKVDNALQSGNSQESVTEQDSKDSTYSLSSTLTLSKADYEKHKVYACEVTHQGLSSPVTKSFNRGEC

SEQ ID NO: 10 - protein, 444 aa, Artificial sequence
  Synthesized
QVQLVQSGAEVKKPGSSVKVSCKASGYSFSSYNIHWVRQAPGQGLEWMGYIAPFQGDSRYNQKFKGRVTITADKSTSTAYMELSSLRSEDTAVYYCARLNRGNSLDYWGQGTLVTVSSASTKGPSVFPLAPCSRSTSESTAALGCLVKDYFPEPVTVSWNSGALTSGVHTFPAVLQSSGLYSLSSVVTVPSSNFGTQTYTCNVDHKPSNTKVDKTVERKCCVECPPCPAPPVAGPSVFLFPPKPKDTLMISRTPEVTCVVVDVSHEDPEVQFNWYVDGVEVHNAKTKPREEQFNSTFRVVSVLTVVHQDWLNGKEYKCKVSNKGLPAPIEKTISKTKGQPREPQVYTLPPSREEMTKNQVSLTCLVKGFYPSDISVEWESNGQPENNYKTTPPMLDSDGSFFLYSKLTVDKSRWQQGNVFSCSVMHEALHNHYTQKSLSLSPGK

SEQ ID NO: 11 - protein, 443 aa, Artificial sequence
  Synthesized
QVQLVQSGAEVKKPGSSVKVSCKASGYSFSSYNIHWVRQAPGQGLEWMGYIAPFQGDSRYNQKFKGRVTITADKSTSTAYMELSSLRSEDTAVYYCARLNRGNSLDYWGQGTLVTVSSASTKGPSVFPLAPCSRSTSESTAALGCLVKDYFPEPVTVSWNSGALTSGVHTFPAVLQSSGLYSLSSVVTVPSSNFGTQTYTCNVDHKPSNTKVDKTVERKCCVECPPCPAPPVAGPSVFLFPPKPKDTLMISRTPEVTCVVVDVSHEDPEVQFNWYVDGVEVHNAKTKPREEQFNSTFRVVSVLTVVHQDWLNGKEYKCKVSNKGLAPIEKTISKTKGQPREPQVYTLPPSREEMTKNQVSLTCLVKGFYPSDISVEWESNGQPENNYKTTPPMLDSDGSFFLYSKLTVDKSRWQQGNVFSCSVMHEALHNHYTQKSLSLSPGK

SEQ ID NO: 12 - protein, 443 aa, Artificial sequence
  Synthesized
QVQLVQSGAEVKKPGSSVKVSCKASGYSFSSYNIHWVRQAPGQGLEWMGYIAPFQGDSRYNQKFKGRVTITADKSTSTAYMELSSLRSEDTAVYYCARLNRGNSLDYWGQGTLVTVSSASTKGPSVFPLAPCSRSTSESTAALGCLVKDYFPEPVTVSWNSGALTSGVHTFPAVLQSSGLYSLSSVVTVPSSNFGTQTYTCNVDHKPSNTKVDKTVERKCCVECPPCPAPPVAGPSVFLFPPKPKDTLMISRTPEVTCVVVDVSHEDPEVQFNWYVDGVEVHNAKTKPREEQFNSTFRVVSVLTVVHQDWLNGKEYKCKVSNKGLGPIEKTISKTKGQPREPQVYTLPPSREEMTKNQVSLTCLVKGFYPSDISVEWESNGQPENNYKTTPPMLDSDGSFFLYSKLTVDKSRWQQGNVFSCSVMHEALHNHYTQKSLSLSPGK

SEQ ID NO: 13 - protein, 442 aa, Artificial sequence
  Synthesized
QVQLVQSGAEVKKPGSSVKVSCKASGYSFSSYNIHWVRQAPGQGLEWMGYIAPFQGDSRYNQKFKGRVTITADKSTSTAYMELSSLRSEDTAVYYCARLNRGNSLDYWGQGTLVTVSSASTKGPSVFPLAPCSRSTSESTAALGCLVKDYFPEPVTVSWNSGALTSGVHTFPAVLQSSGLYSLSSVVTVPSSNFGTQTYTCNVDHKPSNTKVDKTVERKCCVECPPCPAPPVAGPSVFLFPPKPKDTLMISRTPEVTCVVVDVSHEDPEVQFNWYVDGVEVHNAKTKPREEQFNSTFRVVSVLTVVHQDWLNGKEYKCKVSNKGLPIEKTISKTKGQPREPQVYTLPPSREEMTKNQVSLTCLVKGFYPSDISVEWESNGQPENNYKTTPPMLDSDGSFFLYSKLTVDKSRWQQGNVFSCSVMHEALHNHYTQKSLSLSPGK

SEQ ID NO: 14 - protein, 444 aa, Artificial sequence
  Synthesized
QVQLVQSGAEVKKPGSSVKVSCKASGYSFSSYNIHWVRQAPGQGLEWMGYIAPFQGDSRYNQKFKGRVTITADKSTSTAYMELSSLRSEDTAVYYCARLNRGNSLDYWGQGTLVTVSSASTKGPSVFPLAPCSRSTSESTAALGCLVKDYFPEPVTVSWNSGALTSGVHTFPAVLQSSGLYSLSSVVTVPSSNFGTQTYTCNVDHKPSNTKVDKTVERKCCVECPPCPAPPAAGPSVFLFPPKPKDTLMISRTPEVTCVVVDVSHEDPEVQFNWYVDGVEVHNAKTKPREEQFNSTFRVVSVLTVVHQDWLNGKEYKCKVSNKGLPAPIEKTISKTKGQPREPQVYTLPPSREEMTKNQVSLTCLVKGFYPSDISVEWESNGQPENNYKTTPPMLDSDGSFFLYSKLTVDKSRWQQGNVFSCSVMHEALHNHYTQKSLSLSPGK

SEQ ID NO: 15 - protein, 443 aa, Artificial sequence
  Synthesized
QVQLVQSGAEVKKPGSSVKVSCKASGYSFSSYNIHWVRQAPGQGLEWMGYIAPFQGDSRYNQKFKGRVTITADKSTSTAYMELSSLRSEDTAVYYCARLNRGNSLDYWGQGTLVTVSSASTKGPSVFPLAPCSRSTSESTAALGCLVKDYFPEPVTVSWNSGALTSGVHTFPAVLQSSGLYSLSSVVTVPSSNFGTQTYTCNVDHKPSNTKVDKTVERKCCVECPPCPAPPAAGPSVFLFPPKPKDTLMISRTPEVTCVVVDVSHEDPEVQFNWYVDGVEVHNAKTKPREEQFNSTFRVVSVLTVVHQDWLNGKEYKCKVSNKGLAPIEKTISKTKGQPREPQVYTLPPSREEMTKNQVSLTCLVKGFYPSDISVEWESNGQPENNYKTTPPMLDSDGSFFLYSKLTVDKSRWQQGNVFSCSVMHEALHNHYTQKSLSLSPGK

SEQ ID NO: 16 - protein, 443 aa, Artificial sequence
  Synthesized
QVQLVQSGAEVKKPGSSVKVSCKASGYSFSSYNIHWVRQAPGQGLEWMGYIAPFQGDSRYNQKFKGRVTITADKSTSTAYMELSSLRSEDTAVYYCARLNRGNSLDYWGQGTLVTVSSASTKGPSVFPLAPCSRSTSESTAALGCLVKDYFPEPVTVSWNSGALTSGVHTFPAVLQSSGLYSLSSVVTVPSSNFGTQTYTCNVDHKPSNTKVDKTVERKCCVECPPCPAPPAAGPSVFLFPPKPKDTLMISRTPEVTCVVVDVSHEDPEVQFNWYVDGVEVHNAKTKPREEQFNSTFRVVSVLTVVHQDWLNGKEYKCKVSNKGLGPIEKTISKTKGQPREPQVYTLPPSREEMTKNQVSLTCLVKGFYPSDISVEWESNGQPENNYKTTPPMLDSDGSFFLYSKLTVDKSRWQQGNVFSCSVMHEALHNHYTQKSLSLSPGK

SEQ ID NO: 17 - protein, 442 aa, Artificial sequence
  Synthesized
QVQLVQSGAEVKKPGSSVKVSCKASGYSFSSYNIHWVRQAPGQGLEWMGYIAPFQGDSRYNQKFKGRVTITADKSTSTAYMELSSLRSEDTAVYYCARLNRGNSLDYWGQGTLVTVSSASTKGPSVFPLAPCSRSTSESTAALGCLVKDYFPEPVTVSWNSGALTSGVHTFPAVLQSSGLYSLSSVVTVPSSNFGTQTYTCNVDHKPSNTKVDKTVERKCCVECPPCPAPPAAGPSVFLFPPKPKDTLMISRTPEVTCVVVDVSHEDPEVQFNWYVDGVEVHNAKTKPREEQFNSTFRVVSVLTVVHQDWLNGKEYKCKVSNKGLPIEKTISKTKGQPREPQVYTLPPSREEMTKNQVSLTCLVKGFYPSDISVEWESNGQPENNYKTTPPMLDSDGSFFLYSKLTVDKSRWQQGNVFSCSVMHEALHNHYTQKSLSLSPGK

SEQ ID NO: 18 - protein, 445 aa, Artificial sequence
  Synthesized
QVQLVQSGAEVKKPGSSVKVSCKASGYSFSSYNIHWVRQAPGQGLEWMGYIAPFQGDSRYNQKFKGRVTITADKSTSTAYMELSSLRSEDTAVYYCARLNRGNSLDYWGQGTLVTVSSASTKGPSVFPLAPCSRSTSESTAALGCLVKDYFPEPVTVSWNSGALTSGVHTFPAVLQSSGLYSLSSVVTVPSSSLGTKTYTCNVDHKPSNTKVDKRVESKYGPPCPPCPAPEFLGGPSVFLFPPKPKDTLMISRTPEVTCVVVDVSQEDPEVQFNWYVDGVEVHNAKTKPREEQFNSTYRVVSVLTVLHQDWLNGKEYKCKVSNKGLPSSIEKTISKAKGQPREPQVYTLPPSQEEMTKNQVSLTCLVKGFYPSDIAVEWESNGQPENNYKTTPPVLDSDGSFFLYSRLTVDKSRWQEGNVFSCSVMHEALHNHYTQKSLSLSLGK

SEQ ID NO: 19 - protein, 444 aa, Artificial sequence
  Synthesized
QVQLVQSGAEVKKPGSSVKVSCKASGYSFSSYNIHWVRQAPGQGLEWMGYIAPFQGDSRYNQKFKGRVTITADKSTSTAYMELSSLRSEDTAVYYCARLNRGNSLDYWGQGTLVTVSSASTKGPSVFPLAPCSRSTSESTAALGCLVKDYFPEPVTVSWNSGALTSGVHTFPAVLQSSGLYSLSSVVTVPSSSLGTKTYTCNVDHKPSNTKVDKRVESKYGPPCPPCPAPEFLGGPSVFLFPPKPKDTLMISRTPEVTCVVVDVSQEDPEVQFNWYVDGVEVHNAKTKPREEQFNSTYRVVSVLTVLHQDWLNGKEYKCKVSNKGLSSIEKTISKAKGQPREPQVYTLPPSQEEMTKNQVSLTCLVKGFYPSDIAVEWESNGQPENNYKTTPPVLDSDGSFFLYSRLTVDKSRWQEGNVFSCSVMHEALHNHYTQKSLSLSLGK

SEQ ID NO: 20 - protein, 444 aa, Artificial sequence
  Synthesized
QVQLVQSGAEVKKPGSSVKVSCKASGYSFSSYNIHWVRQAPGQGLEWMGYIAPFQGDSRYNQKFKGRVTITADKSTSTAYMELSSLRSEDTAVYYCARLNRGNSLDYWGQGTLVTVSSASTKGPSVFPLAPCSRSTSESTAALGCLVKDYFPEPVTVSWNSGALTSGVHTFPAVLQSSGLYSLSSVVTVPSSSLGTKTYTCNVDHKPSNTKVDKRVESKYGPPCPPCPAPEFLGGPSVFLFPPKPKDTLMISRTPEVTCVVVDVSQEDPEVQFNWYVDGVEVHNAKTKPREEQFNSTYRVVSVLTVLHQDWLNGKEYKCKVSNKGLGSIEKTISKAKGQPREPQVYTLPPSQEEMTKNQVSLTCLVKGFYPSDIAVEWESNGQPENNYKTTPPVLDSDGSFFLYSRLTVDKSRWQEGNVFSCSVMHEALHNHYTQKSLSLSLGK

SEQ ID NO: 21 - protein, 443 aa, Artificial sequence
  Synthesized
QVQLVQSGAEVKKPGSSVKVSCKASGYSFSSYNIHWVRQAPGQGLEWMGYIAPFQGDSRYNQKFKGRVTITADKSTSTAYMELSSLRSEDTAVYYCARLNRGNSLDYWGQGTLVTVSSASTKGPSVFPLAPCSRSTSESTAALGCLVKDYFPEPVTVSWNSGALTSGVHTFPAVLQSSGLYSLSSVVTVPSSSLGTKTYTCNVDHKPSNTKVDKRVESKYGPPCPPCPAPEFLGGPSVFLFPPKPKDTLMISRTPEVTCVVVDVSQEDPEVQFNWYVDGVEVHNAKTKPREEQFNSTYRVVSVLTVLHQDWLNGKEYKCKVSNKGLSIEKTISKAKGQPREPQVYTLPPSQEEMTKNQVSLTCLVKGFYPSDIAVEWESNGQPENNYKTTPPVLDSDGSFFLYSRLTVDKSRWQEGNVFSCSVMHEALHNHYTQKSLSLSLGK

SEQ ID NO: 22 - protein, 445 aa, Artificial sequence
  Synthesized
QVQLVQSGAEVKKPGSSVKVSCKASGYSFSSYNIHWVRQAPGQGLEWMGYIAPFQGDSRYNQKFKGRVTITADKSTSTAYMELSSLRSEDTAVYYCARLNRGNSLDYWGQGTLVTVSSASTKGPSVFPLAPCSRSTSESTAALGCLVKDYFPEPVTVSWNSGALTSGVHTFPAVLQSSGLYSLSSVVTVPSSSLGTKTYTCNVDHKPSNTKVDKRVESKYGPPCPPCPAPEAAGGPSVFLFPPKPKDTLMISRTPEVTCVVVDVSQEDPEVQFNWYVDGVEVHNAKTKPREEQFNSTYRVVSVLTVLHQDWLNGKEYKCKVSNKGLPSSIEKTISKAKGQPREPQVYTLPPSQEEMTKNQVSLTCLVKGFYPSDIAVEWESNGQPENNYKTTPPVLDSDGSFFLYSRLTVDKSRWQEGNVFSCSVMHEALHNHYTQKSLSLSLGK

SEQ ID NO: 23 - protein, 444 aa, Artificial sequence
  Synthesized
QVQLVQSGAEVKKPGSSVKVSCKASGYSFSSYNIHWVRQAPGQGLEWMGYIAPFQGDSRYNQKFKGRVTITADKSTSTAYMELSSLRSEDTAVYYCARLNRGNSLDYWGQGTLVTVSSASTKGPSVFPLAPCSRSTSESTAALGCLVKDYFPEPVTVSWNSGALTSGVHTFPAVLQSSGLYSLSSVVTVPSSSLGTKTYTCNVDHKPSNTKVDKRVESKYGPPCPPCPAPEAAGGPSVFLFPPKPKDTLMISRTPEVTCVVVDVSQEDPEVQFNWYVDGVEVHNAKTKPREEQFNSTYRVVSVLTVLHQDWLNGKEYKCKVSNKGLSSIEKTISKAKGQPREPQVYTLPPSQEEMTKNQVSLTCLVKGFYPSDIAVEWESNGQPENNYKTTPPVLDSDGSFFLYSRLTVDKSRWQEGNVFSCSVMHEALHNHYTQKSLSLSLGK

SEQ ID NO: 24 - protein, 444 aa, Artificial sequence
  Synthesized
QVQLVQSGAEVKKPGSSVKVSCKASGYSFSSYNIHWVRQAPGQGLEWMGYIAPFQGDSRYNQKFKGRVTITADKSTSTAYMELSSLRSEDTAVYYCARLNRGNSLDYWGQGTLVTVSSASTKGPSVFPLAPCSRSTSESTAALGCLVKDYFPEPVTVSWNSGALTSGVHTFPAVLQSSGLYSLSSVVTVPSSSLGTKTYTCNVDHKPSNTKVDKRVESKYGPPCPPCPAPEAAGGPSVFLFPPKPKDTLMISRTPEVTCVVVDVSQEDPEVQFNWYVDGVEVHNAKTKPREEQFNSTYRVVSVLTVLHQDWLNGKEYKCKVSNKGLGSIEKTISKAKGQPREPQVYTLPPSQEEMTKNQVSLTCLVKGFYPSDIAVEWESNGQPENNYKTTPPVLDSDGSFFLYSRLTVDKSRWQEGNVFSCSVMHEALHNHYTQKSLSLSLGK

SEQ ID NO: 25 - protein, 443 aa, Artificial sequence
  Synthesized
QVQLVQSGAEVKKPGSSVKVSCKASGYSFSSYNIHWVRQAPGQGLEWMGYIAPFQGDSRYNQKFKGRVTITADKSTSTAYMELSSLRSEDTAVYYCARLNRGNSLDYWGQGTLVTVSSASTKGPSVFPLAPCSRSTSESTAALGCLVKDYFPEPVTVSWNSGALTSGVHTFPAVLQSSGLYSLSSVVTVPSSSLGTKTYTCNVDHKPSNTKVDKRVESKYGPPCPPCPAPEAAGGPSVFLFPPKPKDTLMISRTPEVTCVVVDVSQEDPEVQFNWYVDGVEVHNAKTKPREEQFNSTYRVVSVLTVLHQDWLNGKEYKCKVSNKGLSIEKTISKAKGQPREPQVYTLPPSQEEMTKNQVSLTCLVKGFYPSDIAVEWESNGQPENNYKTTPPVLDSDGSFFLYSRLTVDKSRWQEGNVFSCSVMHEALHNHYTQKSLSLSLGK

SEQ ID NO: 26 - protein, 450 aa, Artificial sequence
  Synthesized
EVQLVESGGGLVQPGGSLRLSCAASGFNIKDTYIHWVRQAPGKGLEWVARIYPTNGYTRYADSVKGRFTISADTSKNTAYLQMNSLRAEDTAVYYCSRWGGDGFYAMDYWGQGTLVTVSSASTKGPSVFPLAPSSKSTSGGTAALGCLVKDYFPEPVTVSWNSGALTSGVHTFPAVLQSSGLYSLSSVVTVPSSSLGTQTYICNVNHKPSNTKVDKKVEPKSCDKTHTCPPCPAPELLGGPSVFLFPPKPKDTLMISRTPEVTCVVVDVSHEDPEVKFNWYVDGVEVHNAKTKPREEQYNSTYRVVSVLTVLHQDWLNGKEYKCKVSNKALPAPIEKTISKAKGQPREPQVYTLPPSREEMTKNQVSLTCLVKGFYPSDIAVEWESNGQPENNYKTTPPVLDSDGSFFLYSKLTVDKSRWQQGNVFSCSVMHEALHNHYTQKSLSLSPGK

SEQ ID NO: 27 - protein, 449 aa, Artificial sequence
  Synthesized
EVQLVESGGGLVQPGGSLRLSCAASGFNIKDTYIHWVRQAPGKGLEWVARIYPTNGYTRYADSVKGRFTISADTSKNTAYLQMNSLRAEDTAVYYCSRWGGDGFYAMDYWGQGTLVTVSSASTKGPSVFPLAPSSKSTSGGTAALGCLVKDYFPEPVTVSWNSGALTSGVHTFPAVLQSSGLYSLSSVVTVPSSSLGTQTYICNVNHKPSNTKVDKKVEPKSCDKTHTCPPCPAPELLGGPSVFLFPPKPKDTLMISRTPEVTCVVVDVSHEDPEVKFNWYVDGVEVHNAKTKPREEQYNSTYRVVSVLTVLHQDWLNGKEYKCKVSNKALAPIEKTISKAKGQPREPQVYTLPPSREEMTKNQVSLTCLVKGFYPSDIAVEWESNGQPENNYKTTPPVLDSDGSFFLYSKLTVDKSRWQQGNVFSCSVMHEALHNHYTQKSLSLSPGK

SEQ ID NO: 28 - protein, 449 aa, Artificial sequence
  Synthesized
EVQLVESGGGLVQPGGSLRLSCAASGFNIKDTYIHWVRQAPGKGLEWVARIYPTNGYTRYADSVKGRFTISADTSKNTAYLQMNSLRAEDTAVYYCSRWGGDGFYAMDYWGQGTLVTVSSASTKGPSVFPLAPSSKSTSGGTAALGCLVKDYFPEPVTVSWNSGALTSGVHTFPAVLQSSGLYSLSSVVTVPSSSLGTQTYICNVNHKPSNTKVDKKVEPKSCDKTHTCPPCPAPELLGGPSVFLFPPKPKDTLMISRTPEVTCVVVDVSHEDPEVKFNWYVDGVEVHNAKTKPREEQYNSTYRVVSVLTVLHQDWLNGKEYKCKVSNKALGPIEKTISKAKGQPREPQVYTLPPSREEMTKNQVSLTCLVKGFYPSDIAVEWESNGQPENNYKTTPPVLDSDGSFFLYSKLTVDKSRWQQGNVFSCSVMHEALHNHYTQKSLSLSPGK

SEQ ID NO: 29 - protein, 448 aa, Artificial sequence
  Synthesized
EVQLVESGGGLVQPGGSLRLSCAASGFNIKDTYIHWVRQAPGKGLEWVARIYPTNGYTRYADSVKGRFTISADTSKNTAYLQMNSLRAEDTAVYYCSRWGGDGFYAMDYWGQGTLVTVSSASTKGPSVFPLAPSSKSTSGGTAALGCLVKDYFPEPVTVSWNSGALTSGVHTFPAVLQSSGLYSLSSVVTVPSSSLGTQTYICNVNHKPSNTKVDKKVEPKSCDKTHTCPPCPAPELLGGPSVFLFPPKPKDTLMISRTPEVTCVVVDVSHEDPEVKFNWYVDGVEVHNAKTKPREEQYNSTYRVVSVLTVLHQDWLNGKEYKCKVSNKALPIEKTISKAKGQPREPQVYTLPPSREEMTKNQVSLTCLVKGFYPSDIAVEWESNGQPENNYKTTPPVLDSDGSFFLYSKLTVDKSRWQQGNVFSCSVMHEALHNHYTQKSLSLSPGK

SEQ ID NO: 30 - protein, 450 aa, Artificial sequence
  Synthesized
EVQLVESGGGLVQPGGSLRLSCAASGFNIKDTYIHWVRQAPGKGLEWVARIYPTNGYTRYADSVKGRFTISADTSKNTAYLQMNSLRAEDTAVYYCSRWGGDGFYAMDYWGQGTLVTVSSASTKGPSVFPLAPSSKSTSGGTAALGCLVKDYFPEPVTVSWNSGALTSGVHTFPAVLQSSGLYSLSSVVTVPSSSLGTQTYICNVNHKPSNTKVDKKVEPKSCDKTHTCPPCPAPEAAGGPSVFLFPPKPKDTLMISRTPEVTCVVVDVSHEDPEVKFNWYVDGVEVHNAKTKPREEQYNSTYRVVSVLTVLHQDWLNGKEYKCKVSNKALPAPIEKTISKAKGQPREPQVYTLPPSREEMTKNQVSLTCLVKGFYPSDIAVEWESNGQPENNYKTTPPVLDSDGSFFLYSKLTVDKSRWQQGNVFSCSVMHEALHNHYTQKSLSLSPGK

SEQ ID NO: 31 - protein, 449 aa, Artificial sequence
  Synthesized
EVQLVESGGGLVQPGGSLRLSCAASGFNIKDTYIHWVRQAPGKGLEWVARIYPTNGYTRYADSVKGRFTISADTSKNTAYLQMNSLRAEDTAVYYCSRWGGDGFYAMDYWGQGTLVTVSSASTKGPSVFPLAPSSKSTSGGTAALGCLVKDYFPEPVTVSWNSGALTSGVHTFPAVLQSSGLYSLSSVVTVPSSSLGTQTYICNVNHKPSNTKVDKKVEPKSCDKTHTCPPCPAPEAAGGPSVFLFPPKPKDTLMISRTPEVTCVVVDVSHEDPEVKFNWYVDGVEVHNAKTKPREEQYNSTYRVVSVLTVLHQDWLNGKEYKCKVSNKALAPIEKTISKAKGQPREPQVYTLPPSREEMTKNQVSLTCLVKGFYPSDIAVEWESNGQPENNYKTTPPVLDSDGSFFLYSKLTVDKSRWQQGNVFSCSVMHEALHNHYTQKSLSLSPGK

SEQ ID NO: 32 - protein, 449 aa, Artificial sequence
  Synthesized
EVQLVESGGGLVQPGGSLRLSCAASGFNIKDTYIHWVRQAPGKGLEWVARIYPTNGYTRYADSVKGRFTISADTSKNTAYLQMNSLRAEDTAVYYCSRWGGDGFYAMDYWGQGTLVTVSSASTKGPSVFPLAPSSKSTSGGTAALGCLVKDYFPEPVTVSWNSGALTSGVHTFPAVLQSSGLYSLSSVVTVPSSSLGTQTYICNVNHKPSNTKVDKKVEPKSCDKTHTCPPCPAPEAAGGPSVFLFPPKPKDTLMISRTPEVTCVVVDVSHEDPEVKFNWYVDGVEVHNAKTKPREEQYNSTYRVVSVLTVLHQDWLNGKEYKCKVSNKALGPIEKTISKAKGQPREPQVYTLPPSREEMTKNQVSLTCLVKGFYPSDIAVEWESNGQPENNYKTTPPVLDSDGSFFLYSKLTVDKSRWQQGNVFSCSVMHEALHNHYTQKSLSLSPGK

SEQ ID NO: 33 - protein, 448 aa, Artificial sequence
  Synthesized
EVQLVESGGGLVQPGGSLRLSCAASGFNIKDTYIHWVRQAPGKGLEWVARIYPTNGYTRYADSVKGRFTISADTSKNTAYLQMNSLRAEDTAVYYCSRWGGDGFYAMDYWGQGTLVTVSSASTKGPSVFPLAPSSKSTSGGTAALGCLVKDYFPEPVTVSWNSGALTSGVHTFPAVLQSSGLYSLSSVVTVPSSSLGTQTYICNVNHKPSNTKVDKKVEPKSCDKTHTCPPCPAPEAAGGPSVFLFPPKPKDTLMISRTPEVTCVVVDVSHEDPEVKFNWYVDGVEVHNAKTKPREEQYNSTYRVVSVLTVLHQDWLNGKEYKCKVSNKALPIEKTISKAKGQPREPQVYTLPPSREEMTKNQVSLTCLVKGFYPSDIAVEWESNGQPENNYKTTPPVLDSDGSFFLYSKLTVDKSRWQQGNVFSCSVMHEALHNHYTQKSLSLSPGK

SEQ ID NO: 34 - protein, 214 aa, Artificial sequence
  Synthesized
DIQMTQSPSSLSASVGDRVTITCRASQDVNTAVAWYQQKPGKAPKLLIYSASFLYSGVPSRFSGSRSGTDFTLTISSLQPEDFATYYCQQHYTTPPTFGQGTKVEIKRTVAAPSVFIFPPSDEQLKSGTASVVCLLNNFYPREAKVQWKVDNALQSGNSQESVTEQDSKDSTYSLSSTLTLSKADYEKHKVYACEVTHQGLSSPVTKSFNRGEC